European Patent Application EP 4 130 256 A1, published February 8, 2023. Title: ENZYME REACTION SOLUTION FOR CONSTRUCTING SEQUENCING LIBRARY AND USE THEREOF. Applicant: JIANGSU CONQUERS MEDICAL TECHNOLOGY CO., LTD. NANJING VAZYME BIOTECH CO., LTD. The sequence listing filed with the application follows.

SEQUENCE LISTING (1 sequence)

SEQ ID NO: 1 - protein, 212 aa, Vibrio vulnificus
APPSTFSAAKQQAAKIYQDHPITFYCGCDIEWQGKKGIPNLETCGYQVRKSQTRASRIEWEHVVPAWQFGHHRQCWQKGGRKNCSKNDQQFRLMEADLHNLSPAIGEVNGDRSNFNFSQWNGVDGVSYGRCEMQVNFKQRKVMPQTELRGSIARTYLYMSQEYGFQLTKQQQLMQAWNKSYPVDEWECSRDDRIAKIQGNHNPFVQQSCQTQ